European Patent Application EP 4 257 616 A1, published October 11, 2023. Title: Trifunctional fusion protein containing tumor-associated antigen (TAA) antibody and application thereof. Applicant: QURE BIOTECHNOLOGY (SHANGHAI) CO., LTD. Application PCT/CN2021/094631. The sequence listing filed with the application follows.

SEQUENCE LISTING (20 sequences)

SEQ ID NO: 1 - protein, 651 aa, Artificial Sequence
  QD3213
MEFGLSWLFLVAILKGVQCQVQLVQSGAEVKKPGASVKVSCKASGYTFTSYIMHWVRQAPGQGLEWMGYINPYNDGTKYNEKFKGRVTMTRDTSTSTVYMELSSLRSEDTAVYYCARLGFTTRNAMDYWGQGTLVTVSSGGGGSGGGGSGGGGSDIVMTQSPDSLAVSLGERATINCKSSQSLLNSGNQKNYLAWYQQKPGQPPKLLIYGASTRESGVPDRFTGSGSGTDFTLTISSLQAEDVAVYYCQNDHSYPFTFGQGTKLEIKESKYGPPCPPCPAPEFLGGPSVFLFPPKPKDTLMISRTPEVTCVVVDVSQEDPEVQFNWYVDGVEVHNAKTKPREEQFNSTYRVVSVLTVLHQDWLNGKEYKCKVSNKGLPSSIEKTISKAKGQPREPQVYTLPPSQEEMTKNQVSLSCAVKGFYPSDIAVEWESNGQPENNYKTTPPVLDSDGSFFLVSRLTVDKSRWQEGNVFSCSVMHEALHNHYTQKSLSLSLGGGGGSGGGGSGGGGSGGGGSIPPHVQKSVNNDMIVTDNNGAVKFPQLCKFCDVRFSTCDNQKSCMSNCSITSICEKPQEVCVAVWRKNDENITLETVCHDPKLPYHDFILEDAASPKCIMKEKKKPGETFFMCSCSSDECNDNIIFSEEYNTSNPD

SEQ ID NO: 2 - protein, 646 aa, Artificial Sequence
  QD3212
MEFGLSWLFLVAILKGVQCDIKLQQSGAELARPGASVKMSCKTSGYTFTRYTMHWVKQRPGQGLEWIGYINPSRGYTNYNQKFKDKATLTTDKSSSTAYMQLSSLTSEDSAVYYCARYYDDHYCLDYWGQGTTLTVSSVEGGSGGSGGSGGSGGVDDIQLTQSPAIMSASPGEKVTMTCRASSSVSYMNWYQQKSGTSPKRWIYDTSKVASGVPYRFSGSGSGTSYSLTISSMEAEDAATYYCQQWSSNPLTFGAGTKLELKESKYGPPCPPCPAPEFLGGPSVFLFPPKPKDTLMISRTPEVTCVVVDVSQEDPEVQFNWYVDGVEVHNAKTKPREEQFNSTYRVVSVLTVLHQDWLNGKEYKCKVSNKGLPSSIEKTISKAKGQPREPQVYTLPPSQEEMTKNQVSLWCLVKGFYPSDIAVEWESNGQPENNYKTTPPVLDSDGSFFLYSRLTVDKSRWQEGNVFSCSVMHEALHNHYTQKSLSLSLGGGGGSGGGGSGGGGSGGGGSIPPHVQKSVNNDMIVTDNNGAVKFPQLCKFCDVRFSTCDNQKSCMSNCSITSICEKPQEVCVAVWRKNDENITLETVCHDPKLPYHDFILEDAASPKCIMKEKKKPGETFFMCSCSSDECNDNIIFSEEYNTSNPD

SEQ ID NO: 3 - protein, 651 aa, Artificial Sequence
  QD3413
MEFGLSWLFLVAILKGVQCQVQLVQSGAEVKKPGASVKVSCKASGYTFTSYIMHWVRQAPGQGLEWMGYINPYNDGTKYNEKFKGRVTMTRDTSTSTVYMELSSLRSEDTAVYYCARLGFTTRNAMDYWGQGTLVTVSSGGGGSGGGGSGGGGSDIVMTQSPDSLAVSLGERATINCKSSQSLLNSGNQKNYLAWYQQKPGQPPKLLIYGASTRESGVPDRFTGSGSGTDFTLTISSLQAEDVAVYYCQNDHSYPFTFGQGTKLEIKESKYGPPCPPCPAPEFLGGPSVFLFPPKPKDTLMISRTPEVTCVVVDVSQEDPEVQFNWYVDGVEVHNAKTKPREEQFNSTYRVVSVLTVLHQDWLNGKEYKCKVSNKGLPSSIEKTISKAKGQPREPQVYTLPPSQEEMTKNQVSLWCLVKGFYPSDIAVEWESNGQPENNYKTTPPVLDSDGSFFLYSRLTVDKSRWQEGNVFSCSVMHEALHNHYTQKSLSLSLGGGGGSGGGGSGGGGSGGGGSIPPHVQKSVNNDMIVTDNNGAVKFPQLCKFCDVRFSTCDNQKSCMSNCSITSICEKPQEVCVAVWRKNDENITLETVCHDPKLPYHDFILEDAASPKCIMKEKKKPGETFFMCSCSSDECNDNIIFSEEYNTSNPD

SEQ ID NO: 4 - protein, 646 aa, Artificial Sequence
  QD3414
MEFGLSWLFLVAILKGVQCDIKLQQSGAELARPGASVKMSCKTSGYTFTRYTMHWVKQRPGQGLEWIGYINPSRGYTNYNQKFKDKATLTTDKSSSTAYMQLSSLTSEDSAVYYCARYYDDHYCLDYWGQGTTLTVSSVEGGSGGSGGSGGSGGVDDIQLTQSPAIMSASPGEKVTMTCRASSSVSYMNWYQQKSGTSPKRWIYDTSKVASGVPYRFSGSGSGTSYSLTISSMEAEDAATYYCQQWSSNPLTFGAGTKLELKESKYGPPCPPCPAPEFLGGPSVFLFPPKPKDTLMISRTPEVTCVVVDVSQEDPEVQFNWYVDGVEVHNAKTKPREEQFNSTYRVVSVLTVLHQDWLNGKEYKCKVSNKGLPSSIEKTISKAKGQPREPQVYTLPPSQEEMTKNQVSLSCAVKGFYPSDIAVEWESNGQPENNYKTTPPVLDSDGSFFLVSRLTVDKSRWQEGNVFSCSVMHEALHNHYTQKSLSLSLGGGGGSGGGGSGGGGSGGGGSIPPHVQKSVNNDMIVTDNNGAVKFPQLCKFCDVRFSTCDNQKSCMSNCSITSICEKPQEVCVAVWRKNDENITLETVCHDPKLPYHDFILEDAASPKCIMKEKKKPGETFFMCSCSSDECNDNIIFSEEYNTSNPD

SEQ ID NO: 5 - protein, 643 aa, Artificial Sequence
  QD3415
IPPHVQKSVNNDMIVTDNNGAVKFPQLCKFCDVRFSTCDNQKSCMSNCSITSICEKPQEVCVAVWRKNDENITLETVCHDPKLPYHDFILEDAASPKCIMKEKKKPGETFFMCSCSSDECNDNIIFSEEYNTSNPDGGGGSGGGGSGGGGSGGGGSQVQLVQSGAEVKKPGASVKVSCKASGYTFTSYIMHWVRQAPGQGLEWMGYINPYNDGTKYNEKFKGRVTMTRDTSTSTVYMELSSLRSEDTAVYYCARLGFTTRNAMDYWGQGTLVTVSSGGGGSGGGGSGGGGSDIVMTQSPDSLAVSLGERATINCKSSQSLLNSGNQKNYLAWYQQKPGQPPKLLIYGASTRESGVPDRFTGSGSGTDFTLTISSLQAEDVAVYYCQNDHSYPFTFGQGTKLEIKGGGGSGGGGSESKYGPPCPPCPAPEFLGGPSVFLFPPKPKDTLMISRTPEVTCVVVDVSQEDPEVQFNWYVDGVEVHNAKTKPREEQFNSTYRVVSVLTVLHQDWLNGKEYKCKVSNKGLPSSIEKTISKAKGQPREPQVYTLPPSQEEMTKNQVSLSCAVKGFYPSDIAVEWESNGQPENNYKTTPPVLDSDGSFFLVSRLTVDKSRWQEGNVFSCSVMHEALHNHYTQKSLSLSLGK

SEQ ID NO: 6 - protein, 637 aa, Artificial Sequence
  QD3416
IPPHVQKSVNNDMIVTDNNGAVKFPQLCKFCDVRFSTCDNQKSCMSNCSITSICEKPQEVCVAVWRKNDENITLETVCHDPKLPYHDFILEDAASPKCIMKEKKKPGETFFMCSCSSDECNDNIIFSEEYNTSNPDGGGSGGGGSGGGGSGGGGSDIKLQQSGAELARPGASVKMSCKTSGYTFTRYTMHWVKQRPGQGLEWIGYINPSRGYTNYNQKFKDKATLTTDKSSSTAYMQLSSLTSEDSAVYYCARYYDDHYCLDYWGQGTTLTVSSVEGGSGGSGGSGGSGGVDDIQLTQSPAIMSASPGEKVTMTCRASSSVSYMNWYQQKSGTSPKRWIYDTSKVASGVPYRFSGSGSGTSYSLTISSMEAEDAATYYCQQWSSNPLTFGAGTKLELKGGGGSGGGGSESKYGPPCPPCPAPEFLGGPSVFLFPPKPKDTLMISRTPEVTCVVVDVSQEDPEVQFNWYVDGVEVHNAKTKPREEQFNSTYRVVSVLTVLHQDWLNGKEYKCKVSNKGLPSSIEKTISKAKGQPREPQVYTLPPSQEEMTKNQVSLWCLVKGFYPSDIAVEWESNGQPENNYKTTPPVLDSDGSFFLYSRLTVDKSRWQEGNVFSCSVMHEALHNHYTQKSLSLSLGK

SEQ ID NO: 7 - protein, 642 aa, Artificial Sequence
  QD3417
IPPHVQKSVNNDMIVTDNNGAVKFPQLCKFCDVRFSTCDNQKSCMSNCSITSICEKPQEVCVAVWRKNDENITLETVCHDPKLPYHDFILEDAASPKCIMKEKKKPGETFFMCSCSSDECNDNIIFSEEYNTSNPDGGGSGGGGSGGGGSGGGGSQVQLVQSGAEVKKPGASVKVSCKASGYTFTSYIMHWVRQAPGQGLEWMGYINPYNDGTKYNEKFKGRVTMTRDTSTSTVYMELSSLRSEDTAVYYCARLGFTTRNAMDYWGQGTLVTVSSGGGGSGGGGSGGGGSDIVMTQSPDSLAVSLGERATINCKSSQSLLNSGNQKNYLAWYQQKPGQPPKLLIYGASTRESGVPDRFTGSGSGTDFTLTISSLQAEDVAVYYCQNDHSYPFTFGQGTKLEIKGGGGSGGGGSESKYGPPCPPCPAPEFLGGPSVFLFPPKPKDTLMISRTPEVTCVVVDVSQEDPEVQFNWYVDGVEVHNAKTKPREEQFNSTYRVVSVLTVLHQDWLNGKEYKCKVSNKGLPSSIEKTISKAKGQPREPQVYTLPPSQEEMTKNQVSLWCLVKGFYPSDIAVEWESNGQPENNYKTTPPVLDSDGSFFLYSRLTVDKSRWQEGNVFSCSVMHEALHNHYTQKSLSLSLGK

SEQ ID NO: 8 - protein, 637 aa, Artificial Sequence
  QD3418
IPPHVQKSVNNDMIVTDNNGAVKFPQLCKFCDVRFSTCDNQKSCMSNCSITSICEKPQEVCVAVWRKNDENITLETVCHDPKLPYHDFILEDAASPKCIMKEKKKPGETFFMCSCSSDECNDNIIFSEEYNTSNPDGGGSGGGGSGGGGSGGGGSDIKLQQSGAELARPGASVKMSCKTSGYTFTRYTMHWVKQRPGQGLEWIGYINPSRGYTNYNQKFKDKATLTTDKSSSTAYMQLSSLTSEDSAVYYCARYYDDHYCLDYWGQGTTLTVSSVEGGSGGSGGSGGSGGVDDIQLTQSPAIMSASPGEKVTMTCRASSSVSYMNWYQQKSGTSPKRWIYDTSKVASGVPYRFSGSGSGTSYSLTISSMEAEDAATYYCQQWSSNPLTFGAGTKLELKGGGGSGGGGSESKYGPPCPPCPAPEFLGGPSVFLFPPKPKDTLMISRTPEVTCVVVDVSQEDPEVQFNWYVDGVEVHNAKTKPREEQFNSTYRVVSVLTVLHQDWLNGKEYKCKVSNKGLPSSIEKTISKAKGQPREPQVYTLPPSQEEMTKNQVSLSCAVKGFYPSDIAVEWESNGQPENNYKTTPPVLDSDGSFFLVSRLTVDKSRWQEGNVFSCSVMHEALHNHYTQKSLSLSLGK

SEQ ID NO: 9 - protein, 641 aa, Artificial Sequence
  QD3419
IPPHVQKSVNNDMIVTDNNGAVKFPQLCKFCDVRFSTCDNQKSCMSNCSITSICEKPQEVCVAVWRKNDENITLETVCHDPKLPYHDFILEDAASPKCIMKEKKKPGETFFMCSCSSDECNDNIIFSEEYNTSNPDGGGSGGGGSESKYGPPCPPCPAPEFLGGPSVFLFPPKPKDTLMISRTPEVTCVVVDVSQEDPEVQFNWYVDGVEVHNAKTKPREEQFNSTYRVVSVLTVLHQDWLNGKEYKCKVSNKGLPSSIEKTISKAKGQPREPQVYTLPPSQEEMTKNQVSLSCAVKGFYPSDIAVEWESNGQPENNYKTTPPVLDSDGSFFLVSRLTVDKSRWQEGNVFSCSVMHEALHNHYTQKSLSLSLGKGGGSGGGGSGGGGSGGGGSDIVMTQSPDSLAVSLGERATINCKSSQSLLNSGNQKNYLAWYQQKPGQPPKLLIYGASTRESGVPDRFTGSGSGTDFTLTISSLQAEDVAVYYCQNDHSYPFTFGQGTKLEIKGGGGSGGGGSGGGGSQVQLVQSGAEVKKPGASVKVSCKASGYTFTSYIMHWVRQAPGQGLEWMGYINPYNDGTKYNEKFKGRVTMTRDTSTSTVYMELSSLRSEDTAVYYCARLGFTTRNAMDYWGQGTLVTVSS

SEQ ID NO: 10 - protein, 632 aa, Artificial Sequence
  QD3420
IPPHVQKSVNNDMIVTDNNGAVKFPQLCKFCDVRFSTCDNQKSCMSNCSITSICEKPQEVCVAVWRKNDENITLETVCHDPKLPYHDFILEDAASPKCIMKEKKKPGETFFMCSCSSDECNDNIIFSEEYNTSNPDGGGSGGGGSESKYGPPCPPCPAPEFLGGPSVFLFPPKPKDTLMISRTPEVTCVVVDVSQEDPEVQFNWYVDGVEVHNAKTKPREEQFNSTYRVVSVLTVLHQDWLNGKEYKCKVSNKGLPSSIEKTISKAKGQPREPQVYTLPPSQEEMTKNQVSLWCLVKGFYPSDIAVEWESNGQPENNYKTTPPVLDSDGSFFLYSRLTVDKSRWQEGNVFSCSVMHEALHNHYTQKSLSLSLGGGGSGGGGSGGGGSGGGGSDIQLTQSPAIMSASPGEKVTMTCRASSSVSYMNWYQQKSGTSPKRWIYDTSKVASGVPYRFSGSGSGTSYSLTISSMEAEDAATYYCQQWSSNPLTFGAGTKLELKGGGGSGGGGSGGGGSDIKLQQSGAELARPGASVKMSCKTSGYTFTRYTMHWVKQRPGQGLEWIGYINPSRGYTNYNQKFKDKATLTTDKSSSTAYMQLSSLTSEDSAVYYCARYYDDHYCLDYWGQGTTLTVSS

SEQ ID NO: 11 - protein, 661 aa, Artificial Sequence
  QD3421
MEFGLSWLFLVAILKGVQCIPPHVQKSVNNDMIVTDNNGAVKFPQLCKFCDVRFSTCDNQKSCMSNCSITSICEKPQEVCVAVWRKNDENITLETVCHDPKLPYHDFILEDAASPKCIMKEKKKPGETFFMCSCSSDECNDNIIFSEEYNTSNPDGGGGSGGGGSESKYGPPCPPCPAPEFLGGPSVFLFPPKPKDTLMISRTPEVTCVVVDVSQEDPEVQFNWYVDGVEVHNAKTKPREEQFNSTYRVVSVLTVLHQDWLNGKEYKCKVSNKGLPSSIEKTISKAKGQPREPQVYTLPPSQEEMTKNQVSLWCLVKGFYPSDIAVEWESNGQPENNYKTTPPVLDSDGSFFLYSRLTVDKSRWQEGNVFSCSVMHEALHNHYTQKSLSLSLGGGGGSGGGGSGGGGSGGGGSQVQLVQSGAEVKKPGASVKVSCKASGYTFTSYIMHWVRQAPGQGLEWMGYINPYNDGTKYNEKFKGRVTMTRDTSTSTVYMELSSLRSEDTAVYYCARLGFTTRNAMDYWGQGTLVTVSSGGGGSGGGGSGGGGSDIVMTQSPDSLAVSLGERATINCKSSQSLLNSGNQKNYLAWYQQKPGQPPKLLIYGASTRESGVPDRFTGSGSGTDFTLTISSLQAEDVAVYYCQNDHSYPFTFGQGTKLEIK

SEQ ID NO: 12 - protein, 656 aa, Artificial Sequence
  QD3422
MEFGLSWLFLVAILKGVQCIPPHVQKSVNNDMIVTDNNGAVKFPQLCKFCDVRFSTCDNQKSCMSNCSITSICEKPQEVCVAVWRKNDENITLETVCHDPKLPYHDFILEDAASPKCIMKEKKKPGETFFMCSCSSDECNDNIIFSEEYNTSNPDGGGGSGGGGSESKYGPPCPPCPAPEFLGGPSVFLFPPKPKDTLMISRTPEVTCVVVDVSQEDPEVQFNWYVDGVEVHNAKTKPREEQFNSTYRVVSVLTVLHQDWLNGKEYKCKVSNKGLPSSIEKTISKAKGQPREPQVYTLPPSQEEMTKNQVSLSCAVKGFYPSDIAVEWESNGQPENNYKTTPPVLDSDGSFFLVSRLTVDKSRWQEGNVFSCSVMHEALHNHYTQKSLSLSLGGGGGSGGGGSGGGGSGGGGSDIKLQQSGAELARPGASVKMSCKTSGYTFTRYTMHWVKQRPGQGLEWIGYINPSRGYTNYNQKFKDKATLTTDKSSSTAYMQLSSLTSEDSAVYYCARYYDDHYCLDYWGQGTTLTVSSVEGGSGGSGGSGGSGGVDDIQLTQSPAIMSASPGEKVTMTCRASSSVSYMNWYQQKSGTSPKRWIYDTSKVASGVPYRFSGSGSGTSYSLTISSMEAEDAATYYCQQWSSNPLTFGAGTKLELK

SEQ ID NO: 13 - protein, 220 aa, Artificial Sequence
  QD1461
DIVMTQSPDSLAVSLGERATINCKSSQSLLNSGNQKNYLAWYQQKPGQPPKLLIYGASTRESGVPDRFTGSGSGTDFTLTISSLQAEDVAVYYCQNDHSYPFTFGQGTKLEIKRTVAAPSVFIFPPSDEQLKSGTASVVCLLNNFYPREAKVQWKVDNALQSGNSQESVTEQDSKDSTYSLSSTLTLSKADYEKHKVYACEVTHQGLSSPVTKSFNRGEC

SEQ ID NO: 14 - protein, 602 aa, Artificial Sequence
  QD3423
QVQLVQSGAEVKKPGASVKVSCKASGYTFTSYIMHWVRQAPGQGLEWMGYINPYNDGTKYNEKFKGRVTMTRDTSTSTVYMELSSLRSEDTAVYYCARLGFTTRNAMDYWGQGTLVTVSSASTKGPSVFPLAPCSRSTSESTAALGCLVKDYFPEPVTVSWNSGALTSGVHTFPAVLQSSGLYSLSSVVTVPSSSLGTKTYTCNVDHKPSNTKVDKRVESKYGPPCPPCPAPEFLGGPSVFLFPPKPKDTLMISRTPEVTCVVVDVSQEDPEVQFNWYVDGVEVHNAKTKPREEQFNSTYRVVSVLTVLHQDWLNGKEYKCKVSNKGLPSSIEKTISKAKGQPREPQVYTLPPSQEEMTKNQVSLSCAVKGFYPSDIAVEWESNGQPENNYKTTPPVLDSDGSFFLVSRLTVDKSRWQEGNVFSCSVMHEALHNHYTQKSLSLSLGGGGGSGGGGSGGGGSGGGGSIPPHVQKSVNNDMIVTDNNGAVKFPQLCKFCDVRFSTCDNQKSCMSNCSITSICEKPQEVCVAVWRKNDENITLETVCHDPKLPYHDFILEDAASPKCIMKEKKKPGETFFMCSCSSDECNDNIIFSEEYNTSNPD

SEQ ID NO: 15 - protein, 895 aa, Artificial Sequence
  QD3424
DIKLQQSGAELARPGASVKMSCKTSGYTFTRYTMHWVKQRPGQGLEWIGYINPSRGYTNYNQKFKDKATLTTDKSSSTAYMQLSSLTSEDSAVYYCARYYDDHYCLDYWGQGTTLTVSSVEGGSGGSGGSGGSGGVDDIQLTQSPAIMSASPGEKVTMTCRASSSVSYMNWYQQKSGTSPKRWIYDTSKVASGVPYRFSGSGSGTSYSLTISSMEAEDAATYYCQQWSSNPLTFGAGTKLELKGGGGSGGGGSGGGGSGGGGSQVQLVQSGAEVKKPGASVKVSCKASGYTFTSYIMHWVRQAPGQGLEWMGYINPYNDGTKYNEKFKGRVTMTRDTSTSTVYMELSSLRSEDTAVYYCARLGFTTRNAMDYWGQGTLVTVSSGGGGSGGGGSGGGGSDIVMTQSPDSLAVSLGERATINCKSSQSLLNSGNQKNYLAWYQQKPGQPPKLLIYGASTRESGVPDRFTGSGSGTDFTLTISSLQAEDVAVYYCQNDHSYPFTFGQGTKLEIKESKYGPPCPPCPAPEFLGGPSVFLFPPKPKDTLMISRTPEVTCVVVDVSQEDPEVQFNWYVDGVEVHNAKTKPREEQFNSTYRVVSVLTVLHQDWLNGKEYKCKVSNKGLPSSIEKTISKAKGQPREPQVYTLPPSQEEMTKNQVSLWCLVKGFYPSDIAVEWESNGQPENNYKTTPPVLDSDGSFFLYSRLTVDKSRWQEGNVFSCSVMHEALHNHYTQKSLSLSLGGGGGSGGGGSGGGGSGGGGSIPPHVQKSVNNDMIVTDNNGAVKFPQLCKFCDVRFSTCDNQKSCMSNCSITSICEKPQEVCVAVWRKNDENITLETVCHDPKLPYHDFILEDAASPKCIMKEKKKPGETFFMCSCSSDECNDNIIFSEEYNTSNPD

SEQ ID NO: 16 - protein, 136 aa, Artificial Sequence
  TGFbRII(ECD)
IPPHVQKSVNNDMIVTDNNGAVKFPQLCKFCDVRFSTCDNQKSCMSNCSITSICEKPQEVCVAVWRKNDENITLETVCHDPKLPYHDFILEDAASPKCIMKEKKKPGETFFMCSCSSDECNDNIIFSEEYNTSNPD

SEQ ID NO: 17 - protein, 229 aa, Artificial Sequence
  FC-Hole
ESKYGPPCPPCPAPEFLGGPSVFLFPPKPKDTLMISRTPEVTCVVVDVSQEDPEVQFNWYVDGVEVHNAKTKPREEQFNSTYRVVSVLTVLHQDWLNGKEYKCKVSNKGLPSSIEKTISKAKGQPREPQVYTLPPSQEEMTKNQVSLSCAVKGFYPSDIAVEWESNGQPENNYKTTPPVLDSDGSFFLVSRLTVDKSRWQEGNVFSCSVMHEALHNHYTQKSLSLSLGK

SEQ ID NO: 18 - protein, 229 aa, Artificial Sequence
  FC-Knob
ESKYGPPCPPCPAPEFLGGPSVFLFPPKPKDTLMISRTPEVTCVVVDVSQEDPEVQFNWYVDGVEVHNAKTKPREEQFNSTYRVVSVLTVLHQDWLNGKEYKCKVSNKGLPSSIEKTISKAKGQPREPQVYTLPPSQEEMTKNQVSLWCLVKGFYPSDIAVEWESNGQPENNYKTTPPVLDSDGSFFLYSRLTVDKSRWQEGNVFSCSVMHEALHNHYTQKSLSLSLGK

SEQ ID NO: 19 - protein, 119 aa, Artificial Sequence
  OKT3-VH
DIKLQQSGAELARPGASVKMSCKTSGYTFTRYTMHWVKQRPGQGLEWIGYINPSRGYTNYNQKFKDKATLTTDKSSSTAYMQLSSLTSEDSAVYYCARYYDDHYCLDYWGQGTTLTVSS

SEQ ID NO: 20 - protein, 106 aa, Artificial Sequence
  OKT3-VL
DIQLTQSPAIMSASPGEKVTMTCRASSSVSYMNWYQQKSGTSPKRWIYDTSKVASGVPYRFSGSGSGTSYSLTISSMEAEDAATYYCQQWSSNPLTFGAGTKLELK